European Patent Application EP 4 273 225 A1, published November 8, 2023. Title: Recombinant Strain with Modified Gene BBD29_11265 for Producing L-Glutamic Acid, and Method for Constructing the Same and Use Thereof. Applicant: NINGXIA EPPEN BIOTECH CO., LTD. The sequence listing filed with the application follows.

SEQUENCE LISTING (33 sequences)

SEQ ID NO: 1 - DNA, 273 bp, Corynebacterium glutamicum
atggctttaggcggcgcagaactgttaattctttttatcctgtttattctgttcatgggcgggatcgcagcgattgtcatcgttatcgttaagttgacccagcggtctaacagtcgtggtgcctcaactacgtccacaattaacattgatccgagtattcatgctgcattgacagagatcgcagctagggacggggtaccggcgtctagcgtggttaacggtcttctgaacgattacatcaataagcgcaggtactggcctcctacgcaataa

SEQ ID NO: 2 - DNA, 273 bp, Artificial Sequence
  BBD29_11265G70A ORF sequence
atggctttaggcggcgcagaactgttaattctttttatcctgtttattctgttcatgggcgggatcgcaacgattgtcatcgttatcgttaagttgacccagcggtctaacagtcgtggtgcctcaactacgtccacaattaacattgatccgagtattcatgctgcattgacagagatcgcagctagggacggggtaccggcgtctagcgtggttaacggtcttctgaacgattacatcaataagcgcaggtactggcctcctacgcaataa

SEQ ID NO: 3 - protein, 90 aa, Corynebacterium glutamicum
MALGGAELLILFILFILFMGGIAAIVIVIVKLTQRSNSRGASTTSTINIDPSIHAALTEIAARDGVPASSVVNGLLNDYINKRRYWPPTQ

SEQ ID NO: 4 - protein, 90 aa, Artificial Sequence
  mutant protein BBD29_11265A24T
MALGGAELLILFILFILFMGGIATIVIVIVKLTQRSNSRGASTTSTINIDPSIHAALTEIAARDGVPASSVVNGLLNDYINKRRYWPPTQ

SEQ ID NO: 5 - DNA, 56 bp, Artificial Sequence
  Primer P1
cagtgccaagcttgcatgcctgcaggtcgactctagcggtgccagacactgtcaag

SEQ ID NO: 6 - DNA, 30 bp, Artificial Sequence
  Primer P2
acgatgacaatcgttgcgatcccgcccatg

SEQ ID NO: 7 - DNA, 30 bp, Artificial Sequence
  Primer P3
catgggcgggatcgcaacgattgtcatcgt

SEQ ID NO: 8 - DNA, 58 bp, Artificial Sequence
  Primer P4
cagctatgaccatgattacgaattcgagctcggtaccccgtcagcccctgaccgttct

SEQ ID NO: 9 - DNA, 20 bp, Artificial Sequence
  Primer P5
ttttctgactgctctgaacc

SEQ ID NO: 10 - DNA, 20 bp, Artificial Sequence
  Primer P6
gaccgttaaccacgctagac

SEQ ID NO: 11 - DNA, 56 bp, Artificial Sequence
  Primer P7
cagtgccaagcttgcatgcctgcaggtcgactctaggacccgcttgccatacgaag

SEQ ID NO: 12 - DNA, 40 bp, Artificial Sequence
  Primer P8
cccagaacacgacaaaaggtatctactcatctgaagaatc

SEQ ID NO: 13 - DNA, 40 bp, Artificial Sequence
  Primer P9
gattcttcagatgagtagataccttttgtcgtgttctggg

SEQ ID NO: 14 - DNA, 40 bp, Artificial Sequence
  Primer P10
caaaccagagtgcccacgaattattgcgtaggaggccagt

SEQ ID NO: 15 - DNA, 40 bp, Artificial Sequence
  Primer P11
actggcctcctacgcaataattcgtgggcactctggtttg

SEQ ID NO: 16 - DNA, 58 bp, Artificial Sequence
  Primer P12
cagctatgaccatgattacgaattcgagctcggtaccccataagaaacaaccacttcc

SEQ ID NO: 17 - DNA, 20 bp, Artificial Sequence
  Primer P13
gtccaaggtgacggccgcac

SEQ ID NO: 18 - DNA, 20 bp, Artificial Sequence
  Primer P14
tgcgatctctgtcaatgcag

SEQ ID NO: 19 - DNA, 20 bp, Artificial Sequence
  Primer P15
ctgggatagtttcaagcctt

SEQ ID NO: 20 - DNA, 20 bp, Artificial Sequence
  Primer P16
atattcggcccagcagcagc

SEQ ID NO: 21 - DNA, 56 bp, Artificial Sequence
  Primer P17
gcttgcatgcctgcaggtcgactctagaggatccccaccttttgtcgtgttctggg

SEQ ID NO: 22 - DNA, 54 bp, Artificial Sequence
  Primer P18
atcaggctgaaaatcttctctcatccgccaaaacttattgcgtaggaggccagt

SEQ ID NO: 23 - DNA, 56 bp, Artificial Sequence
  Primer P19
cagtgccaagcttgcatgcctgcaggtcgactctaggatttcgccacgccatctac

SEQ ID NO: 24 - DNA, 40 bp, Artificial Sequence
  Primer P20
agccccttttagatggggtggttttctccttaaataacgg

SEQ ID NO: 25 - DNA, 40 bp, Artificial Sequence
  Primer P21
ccgttatttaaggagaaaaccaccccatctaaaaggggct

SEQ ID NO: 26 - DNA, 58 bp, Artificial Sequence
  Primer P22
cagctatgaccatgattacgaattcgagctcggtaccccgagggtgagccgggtgcat

SEQ ID NO: 27 - DNA, 20 bp, Artificial Sequence
  Primer P23
gatttcgccacgccatctac

SEQ ID NO: 28 - DNA, 20 bp, Artificial Sequence
  Primer P24
cgagggtgagccgggtgcat

SEQ ID NO: 29 - DNA, 1533 bp, Artificial Sequence
  DNA fragment BBD29_11265 Up-Down
cagtgccaagcttgcatgcctgcaggtcgactctagcggtgccagacactgtcaagcttgaagaagacgccatccacttatccggtgatcgttgcctttacgttgtgaccaactacaactccgccgaagaagcagccgaatggctcaccgccatcgctttcgattacggactgggccttgccgacatgaacgcggacaccatcctgcttttcggcgatgaagattccgacgctgtcgtccaaatcgatgactggttctcccccgctttctctgcgtacggccttccccacctcctggtggaagtcatgcgcctgaaggattccaaaaccccttatcttcgagtcacacttgctgcagatgactcgaaatttatccaaaccctttacgaaaccgacaacaaacaatggttggtggaaacctcttcctccacaggcacggacgaaacccacgtgaagaccattaatgatgtgctggaacgcatcgagacatggttcaaccaggagactgctgtctaaaccttttgtcgtgttctggggttaaccacccttcggccacctgggatagtttcaagcctttccaggtggccgaagaactaaaagggcataatcactgtatgggttaagtagaaagtgtcattttctgactgctctgaaccccaacaaacactcagcaccgttatttaaggagaaaacatggctttaggcggcgcagaactgttaattctttttatcctgtttattctgttcatgggcgggatcgcaacgattgtcatcgttatcgttaagttgacccagcggtctaacagtcgtggtgcctcaactacgtccacaattaacattgatccgagtattcatgctgcattgacagagatcgcagctagggacggggtaccggcgtctagcgtggttaacggtcttctgaacgattacatcaataagcgcaggtactggcctcctacgcaataacaccccatctaaaaggggctctctggcagatatgctctccggcagaagagcctcttaatccttgttgtacattacacagagcccccaaaagaaccccaaaaacaaaaaactgcccctcaccttcccaaaaggaaagcaaggagcagttttaaactcgttgagtgagtgtgacttaagcgtcaacagcctcggtctcgacgatgttcaccaggcgacggttgcgcttggtggaaaactggacagcgccagtcttcaatgcgaagagagtgtcgtcgccaccgcgaccaacattctcacctgggtggaacttggtgccgcgctgacgaacaaggatctcgcctgcggaaacctgctgaccaccgaaacgcttgacgccaaggcgcttagcctcggaatcacgaccgttgctggagctagatgcacccttcttgtgtgccatgtggtaattccctccttctaaaggaaaaactcatagaaagcccgagggcttacttgattccggttaccttcagaacggtcaggggctgacggggtaccgagctcgaattcgtaatcatggtcatagctg

SEQ ID NO: 30 - DNA, 2004 bp, Artificial Sequence
  Homologous arm fragment 1
cagtgccaagcttgcatgcctgcaggtcgactctaggacccgcttgccatacgaagtcctggagaagatctccacccgcatcaccaacgaagttccagacgtaaaccgcgtggttttggacgtaacctccaagccaccaggaaccatcgaatgggagtaggccttaaatgagccttcgttaagcggcaatcaccttatcggtgattgccgctttcccatttctccgggttttctggaactttttgggcgtatgctgggaatgatcttattattttgatttcagaaagcaggagagaccagatgagcgaaatccttgaaacctactgggcaccccacttcggaaacaccgatgaagccgcagcactcgtttcatacttggcacaagcttccggtgatcctattgaggttcacaccctgttcggggatttaggtttagacggactctctggaaactacaccgacactgagatcgacggctacggcgacgcattcctgctggttgcagcactagcagtgttgatggctgaaaacaaagcatccggcggcgtgaatctgggtgaagttgggggagctgataaatcgatccggctgcatgttgaatccaaggaaaacacccagatcaacaccgcattgaagtactttgcgctttccccagaagaccacgcagcggcagatcgcttcgatgaggatgacctgtctgagcttgccaacttgagtgaagagctgcgcggacagctggactaattgctgcccgtttaaggagtccgattcttcagatgagtagataccttttgtcgtgttctggggttaaccacccttcggccacctgggatagtttcaagcctttccaggtggccgaagaactaaaagggcataatcactgtatgggttaagtagaaagtgtcattttctgactgctctgaaccccaacaaacactcagcaccgttatttaaggagaaaacatggctttaggcggcgcagaactgttaattctttttatcctgtttattctgttcatgggcgggatcgcagcgattgtcatcgttatcgttaagttgacccagcggtctaacagtcgtggtgcctcaactacgtccacaattaacattgatccgagtattcatgctgcattgacagagatcgcagctagggacggggtaccggcgtctagcgtggttaacggtcttctgaacgattacatcaataagcgcaggtactggcctcctacgcaataattcgtgggcactctggtttggttaccaggatgggttagtcattctgatcagcgaattccacgttcacatcgccaattccagagttcacaaccagattcagcattggaccttctagatcagcattgtgggcggtgagatctccaacatcacagcgcgctgtgcccacaccggcggtacaacttaggctcacgggcacatcatcgggcagggtgaccatgacttcgccgatccctgaggtgatttggatgttttgttcctgatccaattgggtgaggtggctgaaatcgaggttcatttcacccacgccagaggtgtagctgctgaggagttcatcgttggtggggatgagattgacatcgccgattccagggtcgtcttcaaagtagatgggatcgatatttgaaataaacaggcctgcgagggcgctcatgacaactccggtaccaactacaccgccgacaatccatggccacacatggcgctttttctgaggcttttgtggagggacttgtacatcccaggtgttgtattggttttgggcaagtggatcccaatgaggcgcttcgggggtttgttgcgcgaagggtgcatagtagccctcaacgggggtgatagtgcttagatctggttggggttgtgggtagagatcttcgtttttcatggtggcatcctcagaaacagtgaattcagtggtgagtagtccgcggggtggaagtggttgtttcttatggggtaccgagctcgaattcgtaatcatggtcatagctg

SEQ ID NO: 31 - DNA, 2004 bp, Artificial Sequence
  Homologous arm fragment 2
cagtgccaagcttgcatgcctgcaggtcgactctaggacccgcttgccatacgaagtcctggagaagatctccacccgcatcaccaacgaagttccagacgtaaaccgcgtggttttggacgtaacctccaagccaccaggaaccatcgaatgggagtaggccttaaatgagccttcgttaagcggcaatcaccttatcggtgattgccgctttcccatttctccgggttttctggaactttttgggcgtatgctgggaatgatcttattattttgatttcagaaagcaggagagaccagatgagcgaaatccttgaaacctactgggcaccccacttcggaaacaccgatgaagccgcagcactcgtttcatacttggcacaagcttccggtgatcctattgaggttcacaccctgttcggggatttaggtttagacggactctctggaaactacaccgacactgagatcgacggctacggcgacgcattcctgctggttgcagcactagcagtgttgatggctgaaaacaaagcatccggcggcgtgaatctgggtgaagttgggggagctgataaatcgatccggctgcatgttgaatccaaggaaaacacccagatcaacaccgcattgaagtactttgcgctttccccagaagaccacgcagcggcagatcgcttcgatgaggatgacctgtctgagcttgccaacttgagtgaagagctgcgcggacagctggactaattgctgcccgtttaaggagtccgattcttcagatgagtagataccttttgtcgtgttctggggttaaccacccttcggccacctgggatagtttcaagcctttccaggtggccgaagaactaaaagggcataatcactgtatgggttaagtagaaagtgtcattttctgactgctctgaaccccaacaaacactcagcaccgttatttaaggagaaaacatggctttaggcggcgcagaactgttaattctttttatcctgtttattctgttcatgggcgggatcgcaacgattgtcatcgttatcgttaagttgacccagcggtctaacagtcgtggtgcctcaactacgtccacaattaacattgatccgagtattcatgctgcattgacagagatcgcagctagggacggggtaccggcgtctagcgtggttaacggtcttctgaacgattacatcaataagcgcaggtactggcctcctacgcaataattcgtgggcactctggtttggttaccaggatgggttagtcattctgatcagcgaattccacgttcacatcgccaattccagagttcacaaccagattcagcattggaccttctagatcagcattgtgggcggtgagatctccaacatcacagcgcgctgtgcccacaccggcggtacaacttaggctcacgggcacatcatcgggcagggtgaccatgacttcgccgatccctgaggtgatttggatgttttgttcctgatccaattgggtgaggtggctgaaatcgaggttcatttcacccacgccagaggtgtagctgctgaggagttcatcgttggtggggatgagattgacatcgccgattccagggtcgtcttcaaagtagatgggatcgatatttgaaataaacaggcctgcgagggcgctcatgacaactccggtaccaactacaccgccgacaatccatggccacacatggcgctttttctgaggcttttgtggagggacttgtacatcccaggtgttgtattggttttgggcaagtggatcccaatgaggcgcttcgggggtttgttgcgcgaagggtgcatagtagccctcaacgggggtgatagtgcttagatctggttggggttgtgggtagagatcttcgtttttcatggtggcatcctcagaaacagtgaattcagtggtgagtagtccgcggggtggaagtggttgtttcttatggggtaccgagctcgaattcgtaatcatggtcatagctg

SEQ ID NO: 32 - DNA, 520 bp, Artificial Sequence
  BBD29_11265 gene and its promoter fragment
gcttgcatgcctgcaggtcgactctagaggatccccaccttttgtcgtgttctggggttaaccacccttcggccacctgggatagtttcaagcctttccaggtggccgaagaactaaaagggcataatcactgtatgggttaagtagaaagtgtcattttctgactgctctgaaccccaacaaacactcagcaccgttatttaaggagaaaacatggctttaggcggcgcagaactgttaattctttttatcctgtttattctgttcatgggcgggatcgcagcgattgtcatcgttatcgttaagttgacccagcggtctaacagtcgtggtgcctcaactacgtccacaattaacattgatccgagtattcatgctgcattgacagagatcgcagctagggacggggtaccggcgtctagcgtggttaacggtcttctgaacgattacatcaataagcgcaggtactggcctcctacgcaataagttttggcggatgagagaagattttcagcctgat

SEQ ID NO: 33 - DNA, 520 bp, Artificial Sequence
  BBD29_11265G70A gene and its promoter fragment
gcttgcatgcctgcaggtcgactctagaggatccccaccttttgtcgtgttctggggttaaccacccttcggccacctgggatagtttcaagcctttccaggtggccgaagaactaaaagggcataatcactgtatgggttaagtagaaagtgtcattttctgactgctctgaaccccaacaaacactcagcaccgttatttaaggagaaaacatggctttaggcggcgcagaactgttaattctttttatcctgtttattctgttcatgggcgggatcgcaacgattgtcatcgttatcgttaagttgacccagcggtctaacagtcgtggtgcctcaactacgtccacaattaacattgatccgagtattcatgctgcattgacagagatcgcagctagggacggggtaccggcgtctagcgtggttaacggtcttctgaacgattacatcaataagcgcaggtactggcctcctacgcaataagttttggcggatgagagaagattttcagcctgat